European Patent Application EP 4 349 350 A1, published April 10, 2024. Title: Bacterial strain, composition, drug for use in combination, and use. Applicant: MOON (GUANGZHOU) BIOTECH CO., LTD. Application EP21935727.4. The sequence listing filed with the application follows.

SEQUENCE LISTING (1 sequence)

SEQ ID NO: 1 - DNA, 1397 bp, Artificial Sequence
agtcgaacgaagttgctctttgtgaagccctcgggtggaactgcgagtatacttagtggcggacgggtgagtaacgcgtgagcaatctgccctgcaatgggggacaacagttggaaacgactgctaataccgcatgagaccacgaaaccgcatggttttgaggtaaaaggatttattcgatgcaggatgagctcgcgtcccattagatagttggtgaggtaacggcccaccaagtcaacgatgggtagccgacctgagagggtgatcggccacactggaactgagacacggtccagactcctacgggaggcagcagtggggaatattgggcaatgggggaaaccctgacccagcaacgccgcgtgagggaagaaggtcttcggattgtaaacctttgtcctatgggacgaaacaaatgacggtaccataggaggaagctccggctaactacgtgccagcagccgcggtaatacgtagggagcaagcgttgtccggaattactgggcgtaaagggtgcgtaggtggctatgtaagtcagatgtgaaagaccggggcttaaccccggggttgcatttgaaactgtgtggcttgagtacaggagagggaagtggaattcctagtgtagcggtgaaatgcgtagatattaggaggaacaccagtggcgaaggcgactttctggactgtaactgacactgaagcacgaaagcgtggggagcaaacaggattagataccctggtagtccacgccgtaaacgatggatactaggtgtggggcccgatagggttccgtgccgaagctaacgcattaagtatcccgcctggggagtacgatcgcaaggttgaaactcaaaggaattgacgggggcccgcacaagcagcggagcatgtggtttaattcgaagcaacgcgaagaaccttaccaaggcttgacatcctctgacgactgtagagatacagtttcccttcggggcagagagacaggtggtgcatggttgtcgtcagctcgtgtcgtgagatgttgggttaagtcccgcaacgagcgcaacccttattgctagttgccagcgcgtaaaggcgggaactctagtgagactgccggggacaactcggaggaaggtggggacgacgtcaaatcatcatgccccttatgtcttgggctacacacgtgctacaatggccggtacaaagggcagcgaacccgtaaggggaagcgaatctcaaaaagccggtcccagttcggattgtgggctgcaacccgcccacatgaagtcggagttgctagtaatcgcgaatcagcatgtcgcggtgaatgcgttcccgggccttgtacacaccgcccgtcacaccacggaagttgggagcacccgaagccagtggcttaaccgtaaggagagagc